European Patent Specification EP 3 741 868 B1, published May 22, 2024. Title: RNA-GUIDED TARGETING OF GENETIC AND EPIGENOMIC REGULATORY PROTEINS TO SPECIFIC GENOMIC LOCI. Applicant: THE GENERAL HOSPITAL CORPORATION. Application PCT/US2014/027335. The sequence listing filed with the application follows.

SEQUENCE LISTING (113 sequences)

SEQ ID NO: 1 - RNA, 262 nt, Artificial Sequence
  Description of Artificial Sequence: Synthetic guide polynucleotide
  modified_base (1)..(20): a, c, u, g, unknown or other and this region may encompass 17-20 nucleotides, wherein some positions may be absent
  modified_base (63)..(262): a, c, u, g, unknown or other and this region may encompass 0-200 nucleotides, wherein some positions may be absent
nnnnnnnnnnnnnnnnnnnnguuuuagagcuagaaauagcaaguuaaaauaaggcuaguccgnnnnnnnnnnnnnnnnnnnnnnnnnnnnnnnnnnnnnnnnnnnnnnnnnnnnnnnnnnnnnnnnnnnnnnnnnnnnnnnnnnnnnnnnnnnnnnnnnnnnnnnnnnnnnnnnnnnnnnnnnnnnnnnnnnnnnnnnnnnnnnnnnnnnnnnnnnnnnnnnnnnnnnnnnnnnnnnnnnnnnnnnnnnnnnnnnnnnnnnn

SEQ ID NO: 2 - RNA, 275 nt, Artificial Sequence
  Description of Artificial Sequence: Synthetic guide polynucleotide
  modified_base (1)..(20): a, c, u, g, unknown or other and this region may encompass 17-20 nucleotides, wherein some positions may be absent
  modified_base (76)..(275): a, c, u, g, unknown or other and this region may encompass 0-200 nucleotides, wherein some positions may be absent
nnnnnnnnnnnnnnnnnnnnguuuuagagcuaugcugaaaagcauagcaaguuaaaauaaggcuaguccguuaucnnnnnnnnnnnnnnnnnnnnnnnnnnnnnnnnnnnnnnnnnnnnnnnnnnnnnnnnnnnnnnnnnnnnnnnnnnnnnnnnnnnnnnnnnnnnnnnnnnnnnnnnnnnnnnnnnnnnnnnnnnnnnnnnnnnnnnnnnnnnnnnnnnnnnnnnnnnnnnnnnnnnnnnnnnnnnnnnnnnnnnnnnnnnnnnnnnnnnnnn

SEQ ID NO: 3 - RNA, 287 nt, Artificial Sequence
  Description of Artificial Sequence: Synthetic guide polynucleotide
  modified_base (1)..(20): a, c, u, g, unknown or other and this region may encompass 17-20 nucleotides, wherein some positions may be absent
  modified_base (88)..(287): a, c, u, g, unknown or other and this region may encompass 0-200 nucleotides, wherein some positions may be absent
nnnnnnnnnnnnnnnnnnnnguuuuagagcuaugcuguuuuggaaacaaaacagcauagcaaguuaaaauaaggcuaguccguuaucnnnnnnnnnnnnnnnnnnnnnnnnnnnnnnnnnnnnnnnnnnnnnnnnnnnnnnnnnnnnnnnnnnnnnnnnnnnnnnnnnnnnnnnnnnnnnnnnnnnnnnnnnnnnnnnnnnnnnnnnnnnnnnnnnnnnnnnnnnnnnnnnnnnnnnnnnnnnnnnnnnnnnnnnnnnnnnnnnnnnnnnnnnnnnnnnnnnnnnnn

SEQ ID NO: 4 - RNA, 296 nt, Artificial Sequence
  Description of Artificial Sequence: Synthetic guide polynucleotide
  modified_base (1)..(20): a, c, u, g, unknown or other and this region may encompass 17-20 nucleotides, wherein some positions may be absent
  modified_base (97)..(296): a, c, u, g, unknown or other and this region may encompass 0-200 nucleotides, wherein some positions may be absent
nnnnnnnnnnnnnnnnnnnnguuuuagagcuagaaauagcaaguuaaaauaaggcuaguccguuaucaacuugaaaaaguggcaccgagucggugcnnnnnnnnnnnnnnnnnnnnnnnnnnnnnnnnnnnnnnnnnnnnnnnnnnnnnnnnnnnnnnnnnnnnnnnnnnnnnnnnnnnnnnnnnnnnnnnnnnnnnnnnnnnnnnnnnnnnnnnnnnnnnnnnnnnnnnnnnnnnnnnnnnnnnnnnnnnnnnnnnnnnnnnnnnnnnnnnnnnnnnnnnnnnnnnnnnnnnnnn

SEQ ID NO: 5 - RNA, 96 nt, Artificial Sequence
  Description of Artificial Sequence: Synthetic guide oligonucleotide
  modified_base (1)..(20): a, c, u, g, unknown or other and this region may encompass 17-20 nucleotides, wherein some positions may be absent
nnnnnnnnnnnnnnnnnnnnguuuaagagcuagaaauagcaaguuuaaauaaggcuaguccguuaucaacuugaaaaaguggcaccgagucggugc

SEQ ID NO: 6 - RNA, 106 nt, Artificial Sequence
  Description of Artificial Sequence: Synthetic guide polynucleotide
  modified_base (1)..(20): a, c, u, g, unknown or other and this region may encompass 17-20 nucleotides, wherein some positions may be absent
nnnnnnnnnnnnnnnnnnnnguuuuagagcuaugcuggaaacagcauagcaaguuuaaauaaggcuaguccguuaucaacuugaaaaaguggcaccgagucggugc

SEQ ID NO: 7 - RNA, 106 nt, Artificial Sequence
  Description of Artificial Sequence: Synthetic guide polynucleotide
  modified_base (1)..(20): a, c, u, g, unknown or other and this region may encompass 17-20 nucleotides, wherein some positions may be absent
nnnnnnnnnnnnnnnnnnnnguuuaagagcuaugcuggaaacagcauagcaaguuuaaauaaggcuaguccguuaucaacuugaaaaaguggcaccgagucggugc

SEQ ID NO: 8 - RNA, 79 nt, Artificial Sequence
  Description of Artificial Sequence: Synthetic guide oligonucleotide
ggaaccauucaaaacagcauagcaaguuaaaauaaggcuaguccguuaucaacuugaaaaaguggcaccgagucggugc

SEQ ID NO: 9 - RNA, 62 nt, Artificial Sequence
  Description of Artificial Sequence: Synthetic guide oligonucleotide
ggagcgagcggagcgguacaguuuuagagcuagaaauagcaaguuaaaauaaggcuaguccg

SEQ ID NO: 10 - RNA, 100 nt, Artificial Sequence
  Description of Artificial Sequence: Synthetic guide polynucleotide
ggagcgagcggagcgguacaguuuuagagcuagaaauagcaaguuaaaauaaggcuaguccguuaucaacuugaaaaaguggcaccgagucggugcuuuu

SEQ ID NO: 11 - protein, 8 aa, Artificial Sequence
  Description of Artificial Sequence: Synthetic nuclear localization signal peptide
PKKKRKVS

SEQ ID NO: 12 - protein, 50 aa, Artificial Sequence
  Description of Artificial Sequence: Synthetic VP64 domain polypeptide
DALDDFDLDMLGSDALDDFDLDMLGSDALDDFDLDMLGSDALDDFDLDML

SEQ ID NO: 13 - protein, 1368 aa, Streptococcus pyogenes
MDKKYSIGLAIGTNSVGWAVITDEYKVPSKKFKVLGNTDRHSIKKNLIGALLFDSGETAEATRLKRTARRRYTRRKNRICYLQEIFSNEMAKVDDSFFHRLEESFLVEEDKKHERHPIFGNIVDEVAYHEKYPTIYHLRKKLVDSTDKADLRLIYLALAHMIKFRGHFLIEGDLNPDNSDVDKLFIQLVQTYNQLFEENPINASGVDAKAILSARLSKSRRLENLIAQLPGEKKNGLFGNLIALSLGLTPNFKSNFDLAEDAKLQLSKDTYDDDLDNLLAQIGDQYADLFLAAKNLSDAILLSDILRVNTEITKAPLSASMIKRYDEHHQDLTLLKALVRQQLPEKYKEIFFDQSKNGYAGYIDGGASQEEFYKFIKPILEKMDGTEELLVKLNREDLLRKQRTFDNGSIPHQIHLGELHAILRRQEDFYPFLKDNREKIEKILTFRIPYYVGPLARGNSRFAWMTRKSEETITPWNFEEVVDKGASAQSFIERMTNFDKNLPNEKVLPKHSLLYEYFTVYNELTKVKYVTEGMRKPAFLSGEQKKAIVDLLFKTNRKVTVKQLKEDYFKKIECFDSVEISGVEDRFNASLGTYHDLLKIIKDKDFLDNEENEDILEDIVLTLTLFEDREMIEERLKTYAHLFDDKVMKQLKRRRYTGWGRLSRKLINGIRDKQSGKTILDFLKSDGFANRNFMQLIHDDSLTFKEDIQKAQVSGQGDSLHEHIANLAGSPAIKKGILQTVKVVDELVKVMGRHKPENIVIEMARENQTTQKGQKNSRERMKRIEEGIKELGSQILKEHPVENTQLQNEKLYLYYLQNGRDMYVDQELDINRLSDYDVDAIVPQSFLKDDSIDNKVLTRSDKNRGKSDNVPSEEVVKKMKNYWRQLLNAKLITQRKFDNLTKAERGGLSELDKAGFIKRQLVETRQITKHVAQILDSRMNTKYDENDKLIREVKVITLKSKLVSDFRKDFQFYKVREINNYHHAHDAYLNAVVGTALIKKYPKLESEFVYGDYKVYDVRKMIAKSEQEIGKATAKYFFYSNIMNFFKTEITLANGEIRKRPLIETNGETGEIVWDKGRDFATVRKVLSMPQVNIVKKTEVQTGGFSKESILPKRNSDKLIARKKDWDPKKYGGFDSPTVAYSVLVVAKVEKGKSKKLKSVKELLGITIMERSSFEKNPIDFLEAKGYKEVKKDLIIKLPKYSLFELENGRKRMLASAGELQKGNELALPSKYVNFLYLASHYEKLKGSPEDNEQKQLFVEQHKHYLDEIIEQISEFSKRVILADANLDKVLSAYNKHRDKPIREQAENIIHLFTLTNLGAPAAFKYFDTTIDRKRYTSTKEVLDATLIHQSITGLYETRIDLSQLGGD

SEQ ID NO: 14 - protein, 4 aa, Artificial Sequence
  Description of Artificial Sequence: Synthetic linker peptide
GGGS

SEQ ID NO: 15 - protein, 5 aa, Artificial Sequence
  Description of Artificial Sequence: Synthetic linker peptide
GGGGS

SEQ ID NO: 16 - DNA, 23 bp, Artificial Sequence
  Description of Artificial Sequence: Synthetic target binding site oligonucleotide
gtgtgcagacggcagtcactagg

SEQ ID NO: 17 - DNA, 23 bp, Artificial Sequence
  Description of Artificial Sequence: Synthetic target binding site oligonucleotide
gagcagcgtcttcgagagtgagg

SEQ ID NO: 18 - DNA, 23 bp, Artificial Sequence
  Description of Artificial Sequence: Synthetic target binding site oligonucleotide
ggtgagtgagtgtgtgcgtgtgg

SEQ ID NO: 19 - DNA, 23 bp, Artificial Sequence
  Description of Artificial Sequence: Synthetic target binding site oligonucleotide
gttggagcggggagaaggccagg

SEQ ID NO: 20 - DNA, 23 bp, Artificial Sequence
  Description of Artificial Sequence: Synthetic target binding site oligonucleotide
gggtggggggagtttgctcctgg

SEQ ID NO: 21 - DNA, 23 bp, Artificial Sequence
  Description of Artificial Sequence: Synthetic target binding site oligonucleotide
ggctttggaaagggggtgggggg

SEQ ID NO: 22 - DNA, 23 bp, Artificial Sequence
  Description of Artificial Sequence: Synthetic target binding site oligonucleotide
ggggcggggtcccggcggggcgg

SEQ ID NO: 23 - DNA, 23 bp, Artificial Sequence
  Description of Artificial Sequence: Synthetic target binding site oligonucleotide
gctcggaggtcgtggcgctgggg

SEQ ID NO: 24 - DNA, 23 bp, Artificial Sequence
  Description of Artificial Sequence: Synthetic target binding site oligonucleotide
gactcaccggccagggcgctcgg

SEQ ID NO: 25 - DNA, 23 bp, Artificial Sequence
  Description of Artificial Sequence: Synthetic target binding site oligonucleotide
ggcgcagcggttaggtggaccgg

SEQ ID NO: 26 - DNA, 23 bp, Artificial Sequence
  Description of Artificial Sequence: Synthetic target binding site oligonucleotide
ggcgcatggctccgccccgccgg

SEQ ID NO: 27 - DNA, 23 bp, Artificial Sequence
  Description of Artificial Sequence: Synthetic target binding site oligonucleotide
gccacgacctccgagctacccgg

SEQ ID NO: 28 - DNA, 23 bp, Artificial Sequence
  Description of Artificial Sequence: Synthetic target binding site oligonucleotide
gcggcgtgagccctcccccttgg

SEQ ID NO: 29 - DNA, 23 bp, Artificial Sequence
  Description of Artificial Sequence: Synthetic target binding site oligonucleotide
ggaggcggggtggagggggtcgg

SEQ ID NO: 30 - DNA, 23 bp, Artificial Sequence
  Description of Artificial Sequence: Synthetic target binding site oligonucleotide
gggctcacgccgcgctccggcgg

SEQ ID NO: 31 - DNA, 23 bp, Artificial Sequence
  Description of Artificial Sequence: Synthetic target binding site oligonucleotide
gaccccctccaccccgcctccgg

SEQ ID NO: 32 - DNA, 23 bp, Artificial Sequence
  Description of Artificial Sequence: Synthetic target binding site oligonucleotide
gagcgcggagccatctggccggg

SEQ ID NO: 33 - DNA, 23 bp, Artificial Sequence
  Description of Artificial Sequence: Synthetic target binding site oligonucleotide
gcgcggcgcggaaggggttaagg

SEQ ID NO: 34 - DNA, 23 bp, Artificial Sequence
  Description of Artificial Sequence: Synthetic target binding site oligonucleotide
gcggcgcggcgcgggccggcggg

SEQ ID NO: 35 - DNA, 23 bp, Artificial Sequence
  Description of Artificial Sequence: Synthetic target binding site oligonucleotide
gccgcgccgccctcccccgccgg

SEQ ID NO: 36 - DNA, 23 bp, Artificial Sequence
  Description of Artificial Sequence: Synthetic target binding site oligonucleotide
gcggttataaccagccaacccgg

SEQ ID NO: 37 - DNA, 23 bp, Artificial Sequence
  Description of Artificial Sequence: Synthetic target binding site oligonucleotide
gtgcgcggagctgttcggaaggg

SEQ ID NO: 38 - DNA, 26 bp, Artificial Sequence
  Description of Artificial Sequence: Synthetic target binding site oligonucleotide
acaccgtgtgcagacggcagtcactg

SEQ ID NO: 39 - DNA, 26 bp, Artificial Sequence
  Description of Artificial Sequence: Synthetic target binding site oligonucleotide
acaccgagcagcgtcttcgagagtgg

SEQ ID NO: 40 - DNA, 26 bp, Artificial Sequence
  Description of Artificial Sequence: Synthetic target binding site oligonucleotide
acaccggtgagtgagtgtgtgcgtgg

SEQ ID NO: 41 - DNA, 26 bp, Artificial Sequence
  Description of Artificial Sequence: Synthetic target binding site oligonucleotide
acaccgttggagcggggagaaggccg

SEQ ID NO: 42 - DNA, 26 bp, Artificial Sequence
  Description of Artificial Sequence: Synthetic target binding site oligonucleotide
acaccgggtggggggagtttgctccg

SEQ ID NO: 43 - DNA, 26 bp, Artificial Sequence
  Description of Artificial Sequence: Synthetic target binding site oligonucleotide
acaccggctttggaaagggggtgggg

SEQ ID NO: 44 - DNA, 26 bp, Artificial Sequence
  Description of Artificial Sequence: Synthetic target binding site oligonucleotide
acaccggggcggggtcccggcggggg

SEQ ID NO: 45 - DNA, 26 bp, Artificial Sequence
  Description of Artificial Sequence: Synthetic target binding site oligonucleotide
acaccgctcggaggtcgtggcgctgg

SEQ ID NO: 46 - DNA, 26 bp, Artificial Sequence
  Description of Artificial Sequence: Synthetic target binding site oligonucleotide
acaccgactcaccggccagggcgctg

SEQ ID NO: 47 - DNA, 26 bp, Artificial Sequence
  Description of Artificial Sequence: Synthetic target binding site oligonucleotide
acaccggcgcagcggttaggtggacg

SEQ ID NO: 48 - DNA, 26 bp, Artificial Sequence
  Description of Artificial Sequence: Synthetic target binding site oligonucleotide
acaccggcgcatggctccgccccgcg

SEQ ID NO: 49 - DNA, 26 bp, Artificial Sequence
  Description of Artificial Sequence: Synthetic target binding site oligonucleotide
acaccgccacgacctccgagctaccg

SEQ ID NO: 50 - DNA, 26 bp, Artificial Sequence
  Description of Artificial Sequence: Synthetic target binding site oligonucleotide
acaccgcggcgtgagccctccccctg

SEQ ID NO: 51 - DNA, 26 bp, Artificial Sequence
  Description of Artificial Sequence: Synthetic target binding site oligonucleotide
acaccggaggcggggtggagggggtg

SEQ ID NO: 52 - DNA, 26 bp, Artificial Sequence
  Description of Artificial Sequence: Synthetic target binding site oligonucleotide
acaccgggctcacgccgcgctccggg

SEQ ID NO: 53 - DNA, 26 bp, Artificial Sequence
  Description of Artificial Sequence: Synthetic target binding site oligonucleotide
acaccgaccccctccaccccgcctcg

SEQ ID NO: 54 - DNA, 26 bp, Artificial Sequence
  Description of Artificial Sequence: Synthetic target binding site oligonucleotide
acaccgagcgcggagccatctggccg

SEQ ID NO: 55 - DNA, 26 bp, Artificial Sequence
  Description of Artificial Sequence: Synthetic target binding site oligonucleotide
acaccgcgcggcgcggaaggggttag

SEQ ID NO: 56 - DNA, 26 bp, Artificial Sequence
  Description of Artificial Sequence: Synthetic target binding site oligonucleotide
acaccgcggcgcggcgcgggccggcg

SEQ ID NO: 57 - DNA, 26 bp, Artificial Sequence
  Description of Artificial Sequence: Synthetic target binding site oligonucleotide
acaccgccgcgccgccctcccccgcg

SEQ ID NO: 58 - DNA, 26 bp, Artificial Sequence
  Description of Artificial Sequence: Synthetic target binding site oligonucleotide
acaccgcggttataaccagccaaccg

SEQ ID NO: 59 - DNA, 26 bp, Artificial Sequence
  Description of Artificial Sequence: Synthetic target binding site oligonucleotide
acaccgtgcgcggagctgttcggaag

SEQ ID NO: 60 - DNA, 26 bp, Artificial Sequence
  Description of Artificial Sequence: Synthetic target binding site oligonucleotide
aaaacagtgactgccgtctgcacacg

SEQ ID NO: 61 - DNA, 26 bp, Artificial Sequence
  Description of Artificial Sequence: Synthetic target binding site oligonucleotide
aaaaccactctcgaagacgctgctcg

SEQ ID NO: 62 - DNA, 26 bp, Artificial Sequence
  Description of Artificial Sequence: Synthetic target binding site oligonucleotide
aaaaccacgcacacactcactcaccg

SEQ ID NO: 63 - DNA, 26 bp, Artificial Sequence
  Description of Artificial Sequence: Synthetic target binding site oligonucleotide
aaaacggccttctccccgctccaacg

SEQ ID NO: 64 - DNA, 26 bp, Artificial Sequence
  Description of Artificial Sequence: Synthetic target binding site oligonucleotide
aaaacggagcaaactccccccacccg

SEQ ID NO: 65 - DNA, 26 bp, Artificial Sequence
  Description of Artificial Sequence: Synthetic target binding site oligonucleotide
aaaaccccaccccctttccaaagccg

SEQ ID NO: 66 - DNA, 26 bp, Artificial Sequence
  Description of Artificial Sequence: Synthetic target binding site oligonucleotide
aaaacccccgccgggaccccgccccg

SEQ ID NO: 67 - DNA, 26 bp, Artificial Sequence
  Description of Artificial Sequence: Synthetic target binding site oligonucleotide
aaaaccagcgccacgacctccgagcg

SEQ ID NO: 68 - DNA, 26 bp, Artificial Sequence
  Description of Artificial Sequence: Synthetic target binding site oligonucleotide
aaaacagcgccctggccggtgagtcg

SEQ ID NO: 69 - DNA, 26 bp, Artificial Sequence
  Description of Artificial Sequence: Synthetic target binding site oligonucleotide
aaaacgtccacctaaccgctgcgccg

SEQ ID NO: 70 - DNA, 26 bp, Artificial Sequence
  Description of Artificial Sequence: Synthetic target binding site oligonucleotide
aaaacgcggggcggagccatgcgccg

SEQ ID NO: 71 - DNA, 26 bp, Artificial Sequence
  Description of Artificial Sequence: Synthetic target binding site oligonucleotide
aaaacggtagctcggaggtcgtggcg

SEQ ID NO: 72 - DNA, 26 bp, Artificial Sequence
  Description of Artificial Sequence: Synthetic target binding site oligonucleotide
aaaacagggggagggctcacgccgcg

SEQ ID NO: 73 - DNA, 26 bp, Artificial Sequence
  Description of Artificial Sequence: Synthetic target binding site oligonucleotide
aaaacaccccctccaccccgcctccg

SEQ ID NO: 74 - DNA, 26 bp, Artificial Sequence
  Description of Artificial Sequence: Synthetic target binding site oligonucleotide
aaaacccggagcgcggcgtgagcccg

SEQ ID NO: 75 - DNA, 26 bp, Artificial Sequence
  Description of Artificial Sequence: Synthetic target binding site oligonucleotide
aaaacgaggcggggtggagggggtcg

SEQ ID NO: 76 - DNA, 26 bp, Artificial Sequence
  Description of Artificial Sequence: Synthetic target binding site oligonucleotide
aaaacggccagatggctccgcgctcg

SEQ ID NO: 77 - DNA, 26 bp, Artificial Sequence
  Description of Artificial Sequence: Synthetic target binding site oligonucleotide
aaaactaaccccttccgcgccgcgcg

SEQ ID NO: 78 - DNA, 26 bp, Artificial Sequence
  Description of Artificial Sequence: Synthetic target binding site oligonucleotide
aaaacgccggcccgcgccgcgccgcg

SEQ ID NO: 79 - DNA, 26 bp, Artificial Sequence
  Description of Artificial Sequence: Synthetic target binding site oligonucleotide
aaaacgcgggggagggcggcgcggcg

SEQ ID NO: 80 - DNA, 26 bp, Artificial Sequence
  Description of Artificial Sequence: Synthetic target binding site oligonucleotide
aaaacggttggctggttataaccgcg

SEQ ID NO: 81 - DNA, 26 bp, Artificial Sequence
  Description of Artificial Sequence: Synthetic target binding site oligonucleotide
aaaacttccgaacagctccgcgcacg

SEQ ID NO: 82 - DNA, 20 bp, Artificial Sequence
  Description of Artificial Sequence: Synthetic primer
tccagatggcacattgtcag

SEQ ID NO: 83 - DNA, 20 bp, Artificial Sequence
  Description of Artificial Sequence: Synthetic primer
agggagcaggaaagtgaggt

SEQ ID NO: 84 - DNA, 20 bp, Artificial Sequence
  Description of Artificial Sequence: Synthetic primer
gcacgtaacctcactttcct

SEQ ID NO: 85 - DNA, 23 bp, Artificial Sequence
  Description of Artificial Sequence: Synthetic primer
cttgctacctctttcctctttct

SEQ ID NO: 86 - DNA, 22 bp, Artificial Sequence
  Description of Artificial Sequence: Synthetic primer
agagaagtcgaggaagagagag

SEQ ID NO: 87 - DNA, 22 bp, Artificial Sequence
  Description of Artificial Sequence: Synthetic primer
cagcagaaagttcatggtttcg

SEQ ID NO: 88 - protein, 130 aa, Enterobacteria phage lambda
MASNFTQFVLVDNGGTGDVTVAPSNFANGVAEWISSNSRSQAYKVTCSVRQSSAQNRKYTIKVEVPKVATQTVGGVELPVAAWRSYLNMELTIPIFATNSDCELIVKAMQGLLKDGNPIPSAIAANSGIY

SEQ ID NO: 89 - protein, 130 aa, Artificial Sequence
  Description of Artificial Sequence: Synthetic lambda bacteriophage MS2 N55K mutant polypeptide
MASNFTQFVLVDNGGTGDVTVAPSNFANGVAEWISSNSRSQAYKVTCSVRQSSAQKRKYTIKVEVPKVATQTVGGVELPVAAWRSYLNMELTIPIFATNSDCELIVKAMQGLLKDGNPIPSAIAANSGIY

SEQ ID NO: 90 - protein, 117 aa, Artificial Sequence
  Description of Artificial Sequence: Synthetic lambda bacteriophage MS2 deltaFG mutant polypeptide
MASNFTQFVLVDNGGTGDVTVAPSNFANGIAEWISSNSRSQAYKVTCSVRQSSAQNRKYTIKVEVPKGAWRSYLNMELTIPIFATNSDCELIVKAMQGLLKDGNPIPSAIAANSGIY

SEQ ID NO: 91 - protein, 262 aa, Artificial Sequence
  Description of Artificial Sequence: Synthetic dimeric MS2 coat polypeptide
MASNFTQFVLVDNGGTGDVTVAPSNFANGVAEWISSNSRSQAYKVTCSVRQSSAQNRKYTIKVEVPKVATQTVGGVELPVAAWRSYLNMELTIPIFATNSDCELIVKAMQGLLKDGNPIPSAIAANSGLYGAMASNFTQFVLVDNGGTGDVTVAPSNFANGVAEWISSNSRSQAYKVTCSVRQSSAQNRKYTIKVEVPKVATQTVGGVELPVAAWRSYLNMELTIPIFATNSDCELIVKAMQGLLKDGNPIPSAIAANSLIN

SEQ ID NO: 92 - protein, 262 aa, Artificial Sequence
  Description of Artificial Sequence: Synthetic dimeric MS2 N55K mutant coat polypeptide
MASNFTQFVLVDNGGTGDVTVAPSNFANGVAEWISSNSRSQAYKVTCSVRQSSAQKRKYTIKVEVPKVATQTVGGVELPVAAWRSYLNMELTIPIFATNSDCELIVKAMQGLLKDGNPIPSAIAANSGLYGAMASNFTQFVLVDNGGTGDVTVAPSNFANGVAEWISSNSRSQAYKVTCSVRQSSAQKRKYTIKVEVPKVATQTVGGVELPVAAWRSYLNMELTIPIFATNSDCELIVKAMQGLLKDGNPIPSAIAANSLIN

SEQ ID NO: 93 - protein, 236 aa, Artificial Sequence
  Description of Artificial Sequence: Synthetic dimeric MS2 deltaFG mutant coat polypeptide
MASNFTQFVLVDNGGTGDVTVAPSNFANGVAEWISSNSRSQAYKVTCSVRQSSAQKRKYTIKVEVPKGAWRSYLNMELTIPIFATNSDCELIVKAMQGLLKDGNPIPSAIAANSGLYGAMASNFTQFVLVDNGGTGDVTVAPSNFANGVAEWISSNSRSQAYKVTCSVRQSSAQKRKYTIKVEVPKGAWRSYLNMELTIPIFATNSDCELIVKAMQGLLKDGNPIPSAIAANSLIN

SEQ ID NO: 94 - protein, 22 aa, Enterobacteria phage lambda
MDAQTRRRERRAEKQAQWKAAN

SEQ ID NO: 95 - protein, 107 aa, Enterobacteria phage lambda
MDAQTRRRERRAEKQAQWKAANPLLVGVSAKPVNRPILSLNRKPKSRVESALNPIDLTVLAEYHKQIESNLQRIERKNQRTWYSKPGERGITCSGRQKIKGKSIPLI

SEQ ID NO: 96 - RNA, 23 nt, Enterobacteria phage lambda
aaacaugaggauuacccaugucg

SEQ ID NO: 97 - RNA, 23 nt, Artificial Sequence
  Description of Artificial Sequence: Synthetic high affinity MS2 binding oligonucleotide
aaacaugaggaucacccaugucg

SEQ ID NO: 98 - RNA, 15 nt, Enterobacteria phage lambda
gcccugaagaagggc

SEQ ID NO: 99 - RNA, 15 nt, Enterobacteria phage lambda
gcccugaaaaagggc

SEQ ID NO: 100 - DNA, 20 bp, Artificial Sequence
  Description of Artificial Sequence: Synthetic truncated Csy4 binding site oligonucleotide
  Description of combined DNA/RNA molecule: Synthetic truncated Csy4 binding site oligonucleotide
gttcactgccgtataggcag

SEQ ID NO: 101 - RNA, 28 nt, Artificial Sequence
  Description of Artificial Sequence: Synthetic Csy4 binding site oligonucleotide
guucacugccguauaggcagcuaagaaa

SEQ ID NO: 102 - RNA, 32 nt, Artificial Sequence
  Description of Artificial Sequence: Synthetic crRNA oligonucleotide
  modified_base (1)..(20): a, c, u, g, unknown or other and this region may encompass 17-20 nucleotides, wherein some positions may be absent
nnnnnnnnnnnnnnnnnnnnguuuuagagcua

SEQ ID NO: 103 - RNA, 42 nt, Artificial Sequence
  Description of Artificial Sequence: Synthetic crRNA oligonucleotide
  modified_base (1)..(20): a, c, u, g, unknown or other and this region may encompass 17-20 nucleotides, wherein some positions may be absent
nnnnnnnnnnnnnnnnnnnnguuuuagagcuaugcuguuuug

SEQ ID NO: 104 - RNA, 36 nt, Artificial Sequence
  Description of Artificial Sequence: Synthetic crRNA oligonucleotide
  modified_base (1)..(20): a, c, u, g, unknown or other and this region may encompass 17-20 nucleotides, wherein some positions may be absent
nnnnnnnnnnnnnnnnnnnnguuuuagagcuaugcu

SEQ ID NO: 105 - RNA, 60 nt, Artificial Sequence
  Description of Artificial Sequence: Synthetic tracrRNA oligonucleotide
uagcaaguuaaaauaaggcuaguccguuaucaacuugaaaaaguggcaccgagucggugc

SEQ ID NO: 106 - RNA, 64 nt, Artificial Sequence
  Description of Artificial Sequence: Synthetic tracrRNA oligonucleotide
agcauagcaaguuaaaauaaggcuaguccguuaucaacuugaaaaaguggcaccgagucggugc

SEQ ID NO: 107 - DNA, 2279 bp, Artificial Sequence
  Description of Artificial Sequence: Synthetic RNA expression vector polynucleotide
  modified_base (331)..(350): a, c, t, g, unknown or other
gacgtcgctagctgtacaaaaaagcaggctttaaaggaaccaattcagtcgactggatccggtaccaaggtcgggcaggaagagggcctatttcccatgattccttcatatttgcatatacgatacaaggctgttagagagataattagaattaatttgactgtaaacacaaagatattagtacaaaatacgtgacgtagaaagtaataatttcttgggtagtttgcagttttaaaattatgttttaaaatggactatcatatgcttaccgtaacttgaaagtatttcgatttcttggctttatatatcttgtggaaaggacgaaacaccnnnnnnnnnnnnnnnnnnnngttttagagctagaaatagcaagttaaaataaggctagtccgttatcaacttgaaaaagtggcaccgagtcggtgctttttttaagcttgggccgctcgaggtacctctctacatatgacatgtgagcaaaaggccagcaaaaggccaggaaccgtaaaaaggccgcgttgctggcgtttttccataggctccgcccccctgacgagcatcacaaaaatcgacgctcaagtcagaggtggcgaaacccgacaggactataaagataccaggcgtttccccctggaagctccctcgtgcgctctcctgttccgaccctgccgcttaccggatacctgtccgcctttctcccttcgggaagcgtggcgctttctcatagctcacgctgtaggtatctcagttcggtgtaggtcgttcgctccaagctgggctgtgtgcacgaaccccccgttcagcccgaccgctgcgccttatccggtaactatcgtcttgagtccaacccggtaagacacgacttatcgccactggcagcagccactggtaacaggattagcagagcgaggtatgtaggcggtgctacagagttcttgaagtggtggcctaactacggctacactagaagaacagtatttggtatctgcgctctgctgaagccagttaccttcggaaaaagagttggtagctcttgatccggcaaacaaaccaccgctggtagcggtggtttttttgtttgcaagcagcagattacgcgcagaaaaaaaggatctcaagaagatcctttgatcttttctacggggtctgacgctcagtggaacgaaaactcacgttaagggattttggtcatgagattatcaaaaaggatcttcacctagatccttttaaattaaaaatgaagttttaaatcaatctaaagtatatatgagtaaacttggtctgacagttaccaatgcttaatcagtgaggcacctatctcagcgatctgtctatttcgttcatccatagttgcctgactccccgtcgtgtagataactacgatacgggagggcttaccatctggccccagtgctgcaatgataccgcgagacccacgctcaccggctccagatttatcagcaataaaccagccagccggaagggccgagcgcagaagtggtcctgcaactttatccgcctccatccagtctattaattgttgccgggaagctagagtaagtagttcgccagttaatagtttgcgcaacgttgttgccattgctacaggcatcgtggtgtcacgctcgtcgtttggtatggcttcattcagctccggttcccaacgatcaaggcgagttacatgatcccccatgttgtgcaaaaaagcggttagctccttcggtcctccgatcgttgtcagaagtaagttggccgcagtgttatcactcatggttatggcagcactgcataattctcttactgtcatgccatccgtaagatgcttttctgtgactggtgagtactcaaccaagtcattctgagaatagtgtatgcggcgaccgagttgctcttgcccggcgtcaatacgggataataccgcgccacatagcagaactttaaaagtgctcatcattggaaaacgttcttcggggcgaaaactctcaaggatcttaccgctgttgagatccagttcgatgtaacccactcgtgcacccaactgatcttcagcatcttttactttcaccagcgtttctgggtgagcaaaaacaggaaggcaaaatgccgcaaaaaagggaataagggcgacacggaaatgttgaatactcatactcttcctttttcaatattattgaagcatttatcagggttattgtctcatgagcggatacatatttgaatgtatttagaaaaataaacaaataggggttccgcgcacatttccccgaaaagtgccacct

SEQ ID NO: 108 - DNA, 7786 bp, Artificial Sequence
  Description of Artificial Sequence: Synthetic CMV-T7-Cas9 D10A/H840A-3xFlag-VP64 polynucleotide
atatgccaagtacgccccctattgacgtcaatgacggtaaatggcccgcctggcattatgcccagtacatgaccttatgggactttcctacttggcagtacatctacgtattagtcatcgctattaccatggtgatgcggttttggcagtacatcaatgggcgtggatagcggtttgactcacggggatttccaagtctccaccccattgacgtcaatgggagtttgttttggcaccaaaatcaacgggactttccaaaatgtcgtaacaactccgccccattgacgcaaatgggcggtaggcgtgtacggtgggaggtctatataagcagagctggtttagtgaaccgtcagatccgctagagatccgcggccgctaatacgactcactatagggagagccgccaccatggataagaaatactcaataggcttagctatcggcacaaatagcgtcggatgggcggtgatcactgatgaatataaggttccgtctaaaaagttcaaggttctgggaaatacagaccgccacagtatcaaaaaaaatcttataggggctcttttatttgacagtggagagacagcggaagcgactcgtctcaaacggacagctcgtagaaggtatacacgtcggaagaatcgtatttgttatctacaggagattttttcaaatgagatggcgaaagtagatgatagtttctttcatcgacttgaagagtcttttttggtggaagaagacaagaagcatgaacgtcatcctatttttggaaatatagtagatgaagttgcttatcatgagaaatatccaactatctatcatctgcgaaaaaaattggtagattctactgataaagcggatttgcgcttaatctatttggccttagcgcatatgattaagtttcgtggtcattttttgattgagggagatttaaatcctgataatagtgatgtggacaaactatttatccagttggtacaaacctacaatcaattatttgaagaaaaccctattaacgcaagtggagtagatgctaaagcgattctttctgcacgattgagtaaatcaagacgattagaaaatctcattgctcagctccccggtgagaagaaaaatggcttatttgggaatctcattgctttgtcattgggtttgacccctaattttaaatcaaattttgatttggcagaagatgctaaattacagctttcaaaagatacttacgatgatgatttagataatttattggcgcaaattggagatcaatatgctgatttgtttttggcagctaagaatttatcagatgctattttactttcagatatcctaagagtaaatactgaaataactaaggctcccctatcagcttcaatgattaaacgctacgatgaacatcatcaagacttgactcttttaaaagctttagttcgacaacaacttccagaaaagtataaagaaatcttttttgatcaatcaaaaaacggatatgcaggttatattgatgggggagctagccaagaagaattttataaatttatcaaaccaattttagaaaaaatggatggtactgaggaattattggtgaaactaaatcgtgaagatttgctgcgcaagcaacggacctttgacaacggctctattccccatcaaattcacttgggtgagctgcatgctattttgagaagacaagaagacttttatccatttttaaaagacaatcgtgagaagattgaaaaaatcttgacttttcgaattccttattatgttggtccattggcgcgtggcaatagtcgttttgcatggatgactcggaagtctgaagaaacaattaccccatggaattttgaagaagttgtcgataaaggtgcttcagctcaatcatttattgaacgcatgacaaactttgataaaaatcttccaaatgaaaaagtactaccaaaacatagtttgctttatgagtattttacggtttataacgaattgacaaaggtcaaatatgttactgaaggaatgcgaaaaccagcatttctttcaggtgaacagaagaaagccattgttgatttactcttcaaaacaaatcgaaaagtaaccgttaagcaattaaaagaagattatttcaaaaaaatagaatgttttgatagtgttgaaatttcaggagttgaagatagatttaatgcttcattaggtacctaccatgatttgctaaaaattattaaagataaagattttttggataatgaagaaaatgaagatatcttagaggatattgttttaacattgaccttatttgaagatagggagatgattgaggaaagacttaaaacatatgctcacctctttgatgataaggtgatgaaacagcttaaacgtcgccgttatactggttggggacgtttgtctcgaaaattgattaatggtattagggataagcaatctggcaaaacaatattagattttttgaaatcagatggttttgccaatcgcaattttatgcagctgatccatgatgatagtttgacatttaaagaagacattcaaaaagcacaagtgtctggacaaggcgatagtttacatgaacatattgcaaatttagctggtagccctgctattaaaaaaggtattttacagactgtaaaagttgttgatgaattggtcaaagtaatggggcggcataagccagaaaatatcgttattgaaatggcacgtgaaaatcagacaactcaaaagggccagaaaaattcgcgagagcgtatgaaacgaatcgaagaaggtatcaaagaattaggaagtcagattcttaaagagcatcctgttgaaaatactcaattgcaaaatgaaaagctctatctctattatctccaaaatggaagagacatgtatgtggaccaagaattagatattaatcgtttaagtgattatgatgtcgatgccattgttccacaaagtttccttaaagacgattcaatagacaataaggtcttaacgcgttctgataaaaatcgtggtaaatcggataacgttccaagtgaagaagtagtcaaaaagatgaaaaactattggagacaacttctaaacgccaagttaatcactcaacgtaagtttgataatttaacgaaagctgaacgtggaggtttgagtgaacttgataaagctggttttatcaaacgccaattggttgaaactcgccaaatcactaagcatgtggcacaaattttggatagtcgcatgaatactaaatacgatgaaaatgataaacttattcgagaggttaaagtgattaccttaaaatctaaattagtttctgacttccgaaaagatttccaattctataaagtacgtgagattaacaattaccatcatgcccatgatgcgtatctaaatgccgtcgttggaactgctttgattaagaaatatccaaaacttgaatcggagtttgtctatggtgattataaagtttatgatgttcgtaaaatgattgctaagtctgagcaagaaataggcaaagcaaccgcaaaatatttcttttactctaatatcatgaacttcttcaaaacagaaattacacttgcaaatggagagattcgcaaacgccctctaatcgaaactaatggggaaactggagaaattgtctgggataaagggcgagattttgccacagtgcgcaaagtattgtccatgccccaagtcaatattgtcaagaaaacagaagtacagacaggcggattctccaaggagtcaattttaccaaaaagaaattcggacaagcttattgctcgtaaaaaagactgggatccaaaaaaatatggtggttttgatagtccaacggtagcttattcagtcctagtggttgctaaggtggaaaaagggaaatcgaagaagttaaaatccgttaaagagttactagggatcacaattatggaaagaagttcctttgaaaaaaatccgattgactttttagaagctaaaggatataaggaagttaaaaaagacttaatcattaaactacctaaatatagtctttttgagttagaaaacggtcgtaaacggatgctggctagtgccggagaattacaaaaaggaaatgagctggctctgccaagcaaatatgtgaattttttatatttagctagtcattatgaaaagttgaagggtagtccagaagataacgaacaaaaacaattgtttgtggagcagcataagcattatttagatgagattattgagcaaatcagtgaattttctaagcgtgttattttagcagatgccaatttagataaagttcttagtgcatataacaaacatagagacaaaccaatacgtgaacaagcagaaaatattattcatttatttacgttgacgaatcttggagctcccgctgcttttaaatattttgatacaacaattgatcgtaaacgatatacgtctacaaaagaagttttagatgccactcttatccatcaatccatcactggtctttatgaaacacgcattgatttgagtcagctaggaggtgacggttctcccaagaagaagaggaaagtctcgagcgactacaaagaccatgacggtgattataaagatcatgacatcgattacaaggatgacgatgacaaggctgcaggaggcggtggaagcgggcgcgccgacgcgctggacgatttcgatctcgacatgctgggttctgatgccctcgatgactttgacctggatatgttgggaagcgacgcattggatgactttgatctggacatgctcggctccgatgctctggacgatttcgatctcgatatgttataaccggtcatcatcaccatcaccattgagtttaaacccgctgatcagcctcgactgtgccttctagttgccagccatctgttgtttgcccctcccccgtgccttccttgaccctggaaggtgccactcccactgtcctttcctaataaaatgaggaaattgcatcgcattgtctgagtaggtgtcattctattctggggggtggggtggggcaggacagcaagggggaggattgggaagacaatagcaggcatgctggggatgcggtgggctctatggcttctgaggcggaaagaaccagctggggctcgataccgtcgacctctagctagagcttggcgtaatcatggtcatagctgtttcctgtgtgaaattgttatccgctcacaattccacacaacatacgagccggaagcataaagtgtaaagcctagggtgcctaatgagtgagctaactcacattaattgcgttgcgctcactgcccgctttccagtcgggaaacctgtcgtgccagctgcattaatgaatcggccaacgcgcggggagaggcggtttgcgtattgggcgctcttccgcttcctcgctcactgactcgctgcgctcggtcgttcggctgcggcgagcggtatcagctcactcaaaggcggtaatacggttatccacagaatcaggggataacgcaggaaagaacatgtgagcaaaaggccagcaaaaggccaggaaccgtaaaaaggccgcgttgctggcgtttttccataggctccgcccccctgacgagcatcacaaaaatcgacgctcaagtcagaggtggcgaaacccgacaggactataaagataccaggcgtttccccctggaagctccctcgtgcgctctcctgttccgaccctgccgcttaccggatacctgtccgcctttctcccttcgggaagcgtggcgctttctcaatgctcacgctgtaggtatctcagttcggtgtaggtcgttcgctccaagctgggctgtgtgcacgaaccccccgttcagcccgaccgctgcgccttatccggtaactatcgtcttgagtccaacccggtaagacacgacttatcgccactggcagcagccactggtaacaggattagcagagcgaggtatgtaggcggtgctacagagttcttgaagtggtggcctaactacggctacactagaaggacagtatttggtatctgcgctctgctgaagccagttaccttcggaaaaagagttggtagctcttgatccggcaaacaaaccaccgctggtagcggtggtttttttgtttgcaagcagcagattacgcgcagaaaaaaaggatctcaagaagatcctttgatcttttctacggggtctgacgctcagtggaacgaaaactcacgttaagggattttggtcatgagattatcaaaaaggatcttcacctagatccttttaaattaaaaatgaagttttaaatcaatctaaagtatatatgagtaaacttggtctgacagttaccaatgcttaatcagtgaggcacctatctcagcgatctgtctatttcgttcatccatagttgcctgactccccgtcgtgtagataactacgatacgggagggcttaccatctggccccagtgctgcaatgataccgcgagacccacgctcaccggctccagatttatcagcaataaaccagccagccggaagggccgagcgcagaagtggtcctgcaactttatccgcctccatccagtctattaattgttgccgggaagctagagtaagtagttcgccagttaatagtttgcgcaacgttgttgccattgctacaggcatcgtggtgtcacgctcgtcgtttggtatggcttcattcagctccggttcccaacgatcaaggcgagttacatgatcccccatgttgtgcaaaaaagcggttagctccttcggtcctccgatcgttgtcagaagtaagttggccgcagtgttatcactcatggttatggcagcactgcataattctcttactgtcatgccatccgtaagatgcttttctgtgactggtgagtactcaaccaagtcattctgagaatagtgtatgcggcgaccgagttgctcttgcccggcgtcaatacgggataataccgcgccacatagcagaactttaaaagtgctcatcattggaaaacgttcttcggggcgaaaactctcaaggatcttaccgctgttgagatccagttcgatgtaacccactcgtgcacccaactgatcttcagcatcttttactttcaccagcgtttctgggtgagcaaaaacaggaaggcaaaatgccgcaaaaaagggaataagggcgacacggaaatgttgaatactcatactcttcctttttcaatattattgaagcatttatcagggttattgtctcatgagcggatacatatttgaatgtatttagaaaaataaacaaataggggttccgcgcacatttccccgaaaagtgccacctgacgtcgacggatcgggagatcgatctcccgatcccctagggtcgactctcagtacaatctgctctgatgccgcatagttaagccagtatctgctccctgcttgtgtgttggaggtcgctgagtagtgcgcgagcaaaatttaagctacaacaaggcaaggcttgaccgacaattgcatgaagaatctgcttagggttaggcgttttgcgctgcttcgcgatgtacgggccagatatacgcgttgacattgattattgactagttattaatagtaatcaattacggggtcattagttcatagcccatatatggagttccgcgttacataacttacggtaaatggcccgcctggctgaccgcccaacgacccccgcccattgacgtcaataatgacgtatgttcccatagtaacgccaatagggactttccattgacgtcaatgggtggactatttacggtaaactgcccacttggcagtacatcaagtgtatcc

SEQ ID NO: 109 - DNA, 7785 bp, Artificial Sequence
  Description of Artificial Sequence: Synthetic MV-T7-Cas9 recoded D10A/H840A-3xFLAG-VP64 polynucleotide
atatgccaagtacgccccctattgacgtcaatgacggtaaatggcccgcctggcattatgcccagtacatgaccttatgggactttcctacttggcagtacatctacgtattagtcatcgctattaccatggtgatgcggttttggcagtacatcaatgggcgtggatagcggtttgactcacggggatttccaagtctccaccccattgacgtcaatgggagtttgttttggcaccaaaatcaacgggactttccaaaatgtcgtaacaactccgccccattgacgcaaatgggcggtaggcgtgtacggtgggaggtctatataagcagagctggtttagtgaaccgtcagatccgctagagatccgcggccgctaatacgactcactatagggagagccgccaccatggataaaaagtattctattggtttagccatcggcactaattccgttggatgggctgtcataaccgatgaatacaaagtaccttcaaagaaatttaaggtgttggggaacacagaccgtcattcgattaaaaagaatcttatcggtgccctcctattcgatagtggcgaaacggcagaggcgactcgcctgaaacgaaccgctcggagaaggtatacacgtcgcaagaaccgaatatgttacttacaagaaatttttagcaatgagatggccaaagttgacgattctttctttcaccgtttggaagagtccttccttgtcgaagaggacaagaaacatgaacggcaccccatctttggaaacatagtagatgaggtggcatatcatgaaaagtacccaacgatttatcacctcagaaaaaagctagttgactcaactgataaagcggacctgaggttaatctacttggctcttgcccatatgataaagttccgtgggcactttctcattgagggtgatctaaatccggacaactcggatgtcgacaaactgttcatccagttagtacaaacctataatcagttgtttgaagagaaccctataaatgcaagtggcgtggatgcgaaggctattcttagcgcccgcctctctaaatcccgacggctagaaaacctgatcgcacaattacccggagagaagaaaaatgggttgttcggtaaccttatagcgctctcactaggcctgacaccaaattttaagtcgaacttcgacttagctgaagatgccaaattgcagcttagtaaggacacgtacgatgacgatctcgacaatctactggcacaaattggagatcagtatgcggacttatttttggctgccaaaaaccttagcgatgcaatcctcctatctgacatactgagagttaatactgagattaccaaggcgccgttatccgcttcaatgatcaaaaggtacgatgaacatcaccaagacttgacacttctcaaggccctagtccgtcagcaactgcctgagaaatataaggaaatattctttgatcagtcgaaaaacgggtacgcaggttatattgacggcggagcgagtcaagaggaattctacaagtttatcaaacccatattagagaagatggatgggacggaagagttgcttgtaaaactcaatcgcgaagatctactgcgaaagcagcggactttcgacaacggtagcattccacatcaaatccacttaggcgaattgcatgctatacttagaaggcaggaggatttttatccgttcctcaaagacaatcgtgaaaagattgagaaaatcctaacctttcgcataccttactatgtgggacccctggcccgagggaactctcggttcgcatggatgacaagaaagtccgaagaaacgattactccatggaattttgaggaagttgtcgataaaggtgcgtcagctcaatcgttcatcgagaggatgaccaactttgacaagaatttaccgaacgaaaaagtattgcctaagcacagtttactttacgagtatttcacagtgtacaatgaactcacgaaagttaagtatgtcactgagggcatgcgtaaacccgcctttctaagcggagaacagaagaaagcaatagtagatctgttattcaagaccaaccgcaaagtgacagttaagcaattgaaagaggactactttaagaaaattgaatgcttcgattctgtcgagatctccggggtagaagatcgatttaatgcgtcacttggtacgtatcatgacctcctaaagataattaaagataaggacttcctggataacgaagagaatgaagatatcttagaagatatagtgttgactcttaccctctttgaagatcgggaaatgattgaggaaagactaaaaacatacgctcacctgttcgacgataaggttatgaaacagttaaagaggcgtcgctatacgggctggggacgattgtcgcggaaacttatcaacgggataagagacaagcaaagtggtaaaactattctcgattttctaaagagcgacggcttcgccaataggaactttatgcagctgatccatgatgactctttaaccttcaaagaggatatacaaaaggcacaggtttccggacaaggggactcattgcacgaacatattgcgaatcttgctggttcgccagccatcaaaaagggcatactccagacagtcaaagtagtggatgagctagttaaggtcatgggacgtcacaaaccggaaaacattgtaatcgagatggcacgcgaaaatcaaacgactcagaaggggcaaaaaaacagtcgagagcggatgaagagaatagaagagggtattaaagaactgggcagccagatcttaaaggagcatcctgtggaaaatacccaattgcagaacgagaaactttacctctattacctacaaaatggaagggacatgtatgttgatcaggaactggacataaaccgtttatctgattacgacgtcgatgccattgtaccccaatcctttttgaaggacgattcaatcgacaataaagtgcttacacgctcggataagaaccgagggaaaagtgacaatgttccaagcgaggaagtcgtaaagaaaatgaagaactattggcggcagctcctaaatgcgaaactgataacgcaaagaaagttcgataacttaactaaagctgagaggggtggcttgtctgaacttgacaaggccggatttattaaacgtcagctcgtggaaacccgccaaatcacaaagcatgttgcacagatactagattcccgaatgaatacgaaatacgacgagaacgataagctgattcgggaagtcaaagtaatcactttaaagtcaaaattggtgtcggacttcagaaaggattttcaattctataaagttagggagataaataactaccaccatgcgcacgacgcttatcttaatgccgtcgtagggaccgcactcattaagaaatacccgaagctagaaagtgagtttgtgtatggtgattacaaagtttatgacgtccgtaagatgatcgcgaaaagcgaacaggagataggcaaggctacagccaaatacttcttttattctaacattatgaatttctttaagacggaaatcactctggcaaacggagagatacgcaaacgacctttaattgaaaccaatggggagacaggtgaaatcgtatgggataagggccgggacttcgcgacggtgagaaaagttttgtccatgccccaagtcaacatagtaaagaaaactgaggtgcagaccggagggttttcaaaggaatcgattcttccaaaaaggaatagtgataagctcatcgctcgtaaaaaggactgggacccgaaaaagtacggtggcttcgatagccctacagttgcctattctgtcctagtagtggcaaaagttgagaagggaaaatccaagaaactgaagtcagtcaaagaattattggggataacgattatggagcgctcgtcttttgaaaagaaccccatcgacttccttgaggcgaaaggttacaaggaagtaaaaaaggatctcataattaaactaccaaagtatagtctgtttgagttagaaaatggccgaaaacggatgttggctagcgccggagagcttcaaaaggggaacgaactcgcactaccgtctaaatacgtgaatttcctgtatttagcgtcccattacgagaagttgaaaggttcacctgaagataacgaacagaagcaactttttgttgagcagcacaaacattatctcgacgaaatcatagagcaaatttcggaattcagtaagagagtcatcctagctgatgccaatctggacaaagtattaagcgcatacaacaagcacagggataaacccatacgtgagcaggcggaaaatattatccatttgtttactcttaccaacctcggcgctccagccgcattcaagtattttgacacaacgatagatcgcaaacgatacacttctaccaaggaggtgctagacgcgacactgattcaccaatccatcacgggattatatgaaactcggatagatttgtcacagcttgggggtgacggatcccccaagaagaagaggaaagtctcgagcgactacaaagaccatgacggtgattataaagatcatgacatcgattacaaggatgacgatgacaaggctgcaggaggcggtggaagcgggcgcgccgacgcgctggacgatttcgatctcgacatgctgggttctgatgccctcgatgactttgacctggatatgttgggaagcgacgcattggatgactttgatctggacatgctcggctccgatgctctggacgatttcgatctcgatatgttataaccggtcatcatcaccatcaccattgagtttaaacccgctgatcagcctcgactgtgccttctagttgccagccatctgttgtttgcccctcccccgtgccttccttgaccctggaaggtgccactcccactgtcctttcctaataaaatgaggaaattgcatcgcattgtctgagtaggtgtcattctattctggggggtggggtggggcaggacagcaagggggaggattgggaagacaatagcaggcatgctggggatgcggtgggctctatggcttctgaggcggaaagaaccagctggggctcgataccgtcgacctctagctagagcttggcgtaatcatggtcatagctgtttcctgtgtgaaattgttatccgctcacaattccacacaacatacgagccggaagcataaagtgtaaagcctagggtgcctaatgagtgagctaactcacattaattgcgttgcgctcactgcccgctttccagtcgggaaacctgtcgtgccagctgcattaatgaatcggccaacgcgcggggagaggcggtttgcgtattgggcgctcttccgcttcctcgctcactgactcgctgcgctcggtcgttcggctgcggcgagcggtatcagctcactcaaaggcggtaatacggttatccacagaatcaggggataacgcaggaaagaacatgtgagcaaaaggccagcaaaaggccaggaaccgtaaaaaggccgcgttgctggcgtttttccataggctccgcccccctgacgagcatcacaaaaatcgacgctcaagtcagaggtggcgaaacccgacaggactataaagataccaggcgtttccccctggaagctccctcgtgcgctctcctgttccgaccctgccgcttaccggatacctgtccgcctttctcccttcgggaagcgtggcgctttctcaatgctcacgctgtaggtatctcagttcggtgtaggtcgttcgctccaagctgggctgtgtgcacgaaccccccgttcagcccgaccgctgcgccttatccggtaactatcgtcttgagtccaacccggtaagacacgacttatcgccactggcagcagccactggtaacaggattagcagagcgaggtatgtaggcggtgctacagagttcttgaagtggtggcctaactacggctacactagaaggacagtatttggtatctgcgctctgctgaagccagttaccttcggaaaaagagttggtagctcttgatccggcaaacaaaccaccgctggtagcggtggtttttttgtttgcaagcagcagattacgcgcagaaaaaaaggatctcaagaagatcctttgatcttttctacggggtctgacgctcagtggaacgaaaactcacgttaagggattttggtcatgagattatcaaaaaggatcttcacctagatccttttaaattaaaaatgaagttttaaatcaatctaaagtatatatgagtaaacttggtctgacagttaccaatgcttaatcagtgaggcacctatctcagcgatctgtctatttcgttcatccatagttgcctgactccccgtcgtgtagataactacgatacgggagggcttaccatctggccccagtgctgcaatgataccgcgagacccacgctcaccggctccagatttatcagcaataaaccagccagccggaagggccgagcgcagaagtggtcctgcaactttatccgcctccatccagtctattaattgttgccgggaagctagagtaagtagttcgccagttaatagtttgcgcaacgttgttgccattgctacaggcatcgtggtgtcacgctcgtcgtttggtatggcttcattcagctccggttcccaacgatcaaggcgagttacatgatcccccatgttgtgcaaaaaagcggttagctccttcggtcctccgatcgttgtcagaagtaagttggccgcagtgttatcactcatggttatggcagcactgcataattctcttactgtcatgccatccgtaagatgcttttctgtgactggtgagtactcaaccaagtcattctgagaatagtgtatgcggcgaccgagttgctcttgcccggcgtcaatacgggataataccgcgccacatagcagaactttaaaagtgctcatcattggaaaacgttcttcggggcgaaaactctcaaggatcttaccgctgttgagatccagttcgatgtaacccactcgtgcacccaactgatcttcagcatcttttactttcaccagcgtttctgggtgagcaaaaacaggaaggcaaaatgccgcaaaaaagggaataagggcgacacggaaatgttgaatactcatactcttcctttttcaatattattgaagcatttatcagggttattgtctcatgagcggatacatatttgaatgtatttagaaaaataaacaaataggggttccgcgcacatttccccgaaaagtgccacctgacgtcgacggatcgggagatcgatctcccgatcccctagggtcgactctcagtacaatctgctctgatgccgcatagttaagccagtatctgctccctgcttgtgtgttggaggtcgctgagtagtgcgcgagcaaaatttaagctacaacaaggcaaggcttgaccgacaattgcatgaagaatctgcttagggttaggcgttttgcgctgcttcgcgatgtacgggccagatatacgcgttgacattgattattgactagttattaatagtaatcaattacggggtcattagttcatagcccatatatggagttccgcgttacataacttacggtaaatggcccgcctggctgaccgcccaacgacccccgcccattgacgtcaataatgacgtatgttcccatagtaacgccaatagggactttccattgacgtcaatgggtggactatttacggtaaactgcccacttggcagtacatcaagtgtatc

SEQ ID NO: 110 - protein, 1461 aa, Artificial Sequence
  Description of Artificial Sequence: Synthetic Cas9-activator polypeptide
MDKKYSIGLAIGTNSVGWAVITDEYKVPSKKFKVLGNTDRHSIKKNLIGALLFDSGETAEATRLKRTARRRYTRRKNRICYLQEIFSNEMAKVDDSFFHRLEESFLVEEDKKHERHPIFGNIVDEVAYHEKYPTIYHLRKKLVDSTDKADLRLIYLALAHMIKFRGHFLIEGDLNPDNSDVDKLFIQLVQTYNQLFEENPINASGVDAKAILSARLSKSRRLENLIAQLPGEKKNGLFGNLIALSLGLTPNFKSNFDLAEDAKLQLSKDTYDDDLDNLLAQIGDQYADLFLAAKNLSDAILLSDILRVNTEITKAPLSASMIKRYDEHHQDLTLLKALVRQQLPEKYKEIFFDQSKNGYAGYIDGGASQEEFYKFIKPILEKMDGTEELLVKLNREDLLRKQRTFDNGSIPHQIHLGELHAILRRQEDFYPFLKDNREKIEKILTFRIPYYVGPLARGNSRFAWMTRKSEETITPWNFEEVVDKGASAQSFIERMTNFDKNLPNEKVLPKHSLLYEYFTVYNELTKVKYVTEGMRKPAFLSGEQKKAIVDLLFKTNRKVTVKQLKEDYFKKIECFDSVEISGVEDRFNASLGTYHDLLKIIKDKDFLDNEENEDILEDIVLTLTLFEDREMIEERLKTYAHLFDDKVMKQLKRRRYTGWGRLSRKLINGIRDKQSGKTILDFLKSDGFANRNFMQLIHDDSLTFKEDIQKAQVSGQGDSLHEHIANLAGSPAIKKGILQTVKVVDELVKVMGRHKPENIVIEMARENQTTQKGQKNSRERMKRIEEGIKELGSQILKEHPVENTQLQNEKLYLYYLQNGRDMYVDQELDINRLSDYDVDAIVPQSFLKDDSIDNKVLTRSDKNRGKSDNVPSEEVVKKMKNYWRQLLNAKLITQRKFDNLTKAERGGLSELDKAGFIKRQLVETRQITKHVAQILDSRMNTKYDENDKLIREVKVITLKSKLVSDFRKDFQFYKVREINNYHHAHDAYLNAVVGTALIKKYPKLESEFVYGDYKVYDVRKMIAKSEQEIGKATAKYFFYSNIMNFFKTEITLANGEIRKRPLIETNGETGEIVWDKGRDFATVRKVLSMPQVNIVKKTEVQTGGFSKESILPKRNSDKLIARKKDWDPKKYGGFDSPTVAYSVLVVAKVEKGKSKKLKSVKELLGITIMERSSFEKNPIDFLEAKGYKEVKKDLIIKLPKYSLFELENGRKRMLASAGELQKGNELALPSKYVNFLYLASHYEKLKGSPEDNEQKQLFVEQHKHYLDEIIEQISEFSKRVILADANLDKVLSAYNKHRDKPIREQAENIIHLFTLTNLGAPAAFKYFDTTIDRKRYTSTKEVLDATLIHQSITGLYETRIDLSQLGGDGSPKKKRKVSSDYKDHDGDYKDHDIDYKDDDDKAAGGGGSGRADALDDFDLDMLGSDALDDFDLDMLGSDALDDFDLDMLGSDALDDFDLDML

SEQ ID NO: 111 - protein, 1527 aa, Artificial Sequence
  Description of Artificial Sequence: Synthetic dCas9-NLS-3xFLAG-HP1alpha polypeptide
MDKKYSIGLAIGTNSVGWAVITDEYKVPSKKFKVLGNTDRHSIKKNLIGALLFDSGETAEATRLKRTARRRYTRRKNRICYLQEIFSNEMAKVDDSFFHRLEESFLVEEDKKHERHPIFGNIVDEVAYHEKYPTIYHLRKKLVDSTDKADLRLIYLALAHMIKFRGHFLIEGDLNPDNSDVDKLFIQLVQTYNQLFEENPINASGVDAKAILSARLSKSRRLENLIAQLPGEKKNGLFGNLIALSLGLTPNFKSNFDLAEDAKLQLSKDTYDDDLDNLLAQIGDQYADLFLAAKNLSDAILLSDILRVNTEITKAPLSASMIKRYDEHHQDLTLLKALVRQQLPEKYKEIFFDQSKNGYAGYIDGGASQEEFYKFIKPILEKMDGTEELLVKLNREDLLRKQRTFDNGSIPHQIHLGELHAILRRQEDFYPFLKDNREKIEKILTFRIPYYVGPLARGNSRFAWMTRKSEETITPWNFEEVVDKGASAQSFIERMTNFDKNLPNEKVLPKHSLLYEYFTVYNELTKVKYVTEGMRKPAFLSGEQKKAIVDLLFKTNRKVTVKQLKEDYFKKIECFDSVEISGVEDRFNASLGTYHDLLKIIKDKDFLDNEENEDILEDIVLTLTLFEDREMIEERLKTYAHLFDDKVMKQLKRRRYTGWGRLSRKLINGIRDKQSGKTILDFLKSDGFANRNFMQLIHDDSLTFKEDIQKAQVSGQGDSLHEHIANLAGSPAIKKGILQTVKVVDELVKVMGRHKPENIVIEMARENQTTQKGQKNSRERMKRIEEGIKELGSQILKEHPVENTQLQNEKLYLYYLQNGRDMYVDQELDINRLSDYDVDAIVPQSFLKDDSIDNKVLTRSDKNRGKSDNVPSEEVVKKMKNYWRQLLNAKLITQRKFDNLTKAERGGLSELDKAGFIKRQLVETRQITKHVAQILDSRMNTKYDENDKLIREVKVITLKSKLVSDFRKDFQFYKVREINNYHHAHDAYLNAVVGTALIKKYPKLESEFVYGDYKVYDVRKMIAKSEQEIGKATAKYFFYSNIMNFFKTEITLANGEIRKRPLIETNGETGEIVWDKGRDFATVRKVLSMPQVNIVKKTEVQTGGFSKESILPKRNSDKLIARKKDWDPKKYGGFDSPTVAYSVLVVAKVEKGKSKKLKSVKELLGITIMERSSFEKNPIDFLEAKGYKEVKKDLIIKLPKYSLFELENGRKRMLASAGELQKGNELALPSKYVNFLYLASHYEKLKGSPEDNEQKQLFVEQHKHYLDEIIEQISEFSKRVILADANLDKVLSAYNKHRDKPIREQAENIIHLFTLTNLGAPAAFKYFDTTIDRKRYTSTKEVLDATLIHQSITGLYETRIDLSQLGGDGSPKKKRKVSSDYKDHDGDYKDHDIDYKDDDDKAAGGGGSMKEGENNKPREKSESNKRKSNFSNSADDIKSKKKREQSNDIARGFERGLEPEKIIGATDSCGDLMFLMKWKDTDEADLVLAKEANVKCPQIVIAFYEERLTWHAYPEDAENKEKETAKS

SEQ ID NO: 112 - protein, 1521 aa, Artificial Sequence
  Description of Artificial Sequence: Synthetic dCas9-NLS-3xFLAG-HP1beta polypeptide
MDKKYSIGLAIGTNSVGWAVITDEYKVPSKKFKVLGNTDRHSIKKNLIGALLFDSGETAEATRLKRTARRRYTRRKNRICYLQEIFSNEMAKVDDSFFHRLEESFLVEEDKKHERHPIFGNIVDEVAYHEKYPTIYHLRKKLVDSTDKADLRLIYLALAHMIKFRGHFLIEGDLNPDNSDVDKLFIQLVQTYNQLFEENPINASGVDAKAILSARLSKSRRLENLIAQLPGEKKNGLFGNLIALSLGLTPNFKSNFDLAEDAKLQLSKDTYDDDLDNLLAQIGDQYADLFLAAKNLSDAILLSDILRVNTEITKAPLSASMIKRYDEHHQDLTLLKALVRQQLPEKYKEIFFDQSKNGYAGYIDGGASQEEFYKFIKPILEKMDGTEELLVKLNREDLLRKQRTFDNGSIPHQIHLGELHAILRRQEDFYPFLKDNREKIEKILTFRIPYYVGPLARGNSRFAWMTRKSEETITPWNFEEVVDKGASAQSFIERMTNFDKNLPNEKVLPKHSLLYEYFTVYNELTKVKYVTEGMRKPAFLSGEQKKAIVDLLFKTNRKVTVKQLKEDYFKKIECFDSVEISGVEDRFNASLGTYHDLLKIIKDKDFLDNEENEDILEDIVLTLTLFEDREMIEERLKTYAHLFDDKVMKQLKRRRYTGWGRLSRKLINGIRDKQSGKTILDFLKSDGFANRNFMQLIHDDSLTFKEDIQKAQVSGQGDSLHEHIANLAGSPAIKKGILQTVKVVDELVKVMGRHKPENIVIEMARENQTTQKGQKNSRERMKRIEEGIKELGSQILKEHPVENTQLQNEKLYLYYLQNGRDMYVDQELDINRLSDYDVDAIVPQSFLKDDSIDNKVLTRSDKNRGKSDNVPSEEVVKKMKNYWRQLLNAKLITQRKFDNLTKAERGGLSELDKAGFIKRQLVETRQITKHVAQILDSRMNTKYDENDKLIREVKVITLKSKLVSDFRKDFQFYKVREINNYHHAHDAYLNAVVGTALIKKYPKLESEFVYGDYKVYDVRKMIAKSEQEIGKATAKYFFYSNIMNFFKTEITLANGEIRKRPLIETNGETGEIVWDKGRDFATVRKVLSMPQVNIVKKTEVQTGGFSKESILPKRNSDKLIARKKDWDPKKYGGFDSPTVAYSVLVVAKVEKGKSKKLKSVKELLGITIMERSSFEKNPIDFLEAKGYKEVKKDLIIKLPKYSLFELENGRKRMLASAGELQKGNELALPSKYVNFLYLASHYEKLKGSPEDNEQKQLFVEQHKHYLDEIIEQISEFSKRVILADANLDKVLSAYNKHRDKPIREQAENIIHLFTLTNLGAPAAFKYFDTTIDRKRYTSTKEVLDATLIHQSITGLYETRIDLSQLGGDGSPKKKRKVSSDYKDHDGDYKDHDIDYKDDDDKAAGGGGSTAHETDKSEGGKRKADSDSEDKGEESKPKKKKEESEKPRGFARGLEPERIIGATDSSGELMFLMKWKNSDEADLVPAKEANVKCPQVVISFYEERLTWHSYPSEDDDKKDDKN

SEQ ID NO: 113 - protein, 2126 aa, Artificial Sequence
  Description of Artificial Sequence: Synthetic dCas9-3xFLAG-TET1CD polypeptide
MDKKYSIGLAIGTNSVGWAVITDEYKVPSKKFKVLGNTDRHSIKKNLIGALLFDSGETAEATRLKRTARRRYTRRKNRICYLQEIFSNEMAKVDDSFFHRLEESFLVEEDKKHERHPIFGNIVDEVAYHEKYPTIYHLRKKLVDSTDKADLRLIYLALAHMIKFRGHFLIEGDLNPDNSDVDKLFIQLVQTYNQLFEENPINASGVDAKAILSARLSKSRRLENLIAQLPGEKKNGLFGNLIALSLGLTPNFKSNFDLAEDAKLQLSKDTYDDDLDNLLAQIGDQYADLFLAAKNLSDAILLSDILRVNTEITKAPLSASMIKRYDEHHQDLTLLKALVRQQLPEKYKEIFFDQSKNGYAGYIDGGASQEEFYKFIKPILEKMDGTEELLVKLNREDLLRKQRTFDNGSIPHQIHLGELHAILRRQEDFYPFLKDNREKIEKILTFRIPYYVGPLARGNSRFAWMTRKSEETITPWNFEEVVDKGASAQSFIERMTNFDKNLPNEKVLPKHSLLYEYFTVYNELTKVKYVTEGMRKPAFLSGEQKKAIVDLLFKTNRKVTVKQLKEDYFKKIECFDSVEISGVEDRFNASLGTYHDLLKIIKDKDFLDNEENEDILEDIVLTLTLFEDREMIEERLKTYAHLFDDKVMKQLKRRRYTGWGRLSRKLINGIRDKQSGKTILDFLKSDGFANRNFMQLIHDDSLTFKEDIQKAQVSGQGDSLHEHIANLAGSPAIKKGILQTVKVVDELVKVMGRHKPENIVIEMARENQTTQKGQKNSRERMKRIEEGIKELGSQILKEHPVENTQLQNEKLYLYYLQNGRDMYVDQELDINRLSDYDVDAIVPQSFLKDDSIDNKVLTRSDKNRGKSDNVPSEEVVKKMKNYWRQLLNAKLITQRKFDNLTKAERGGLSELDKAGFIKRQLVETRQITKHVAQILDSRMNTKYDENDKLIREVKVITLKSKLVSDFRKDFQFYKVREINNYHHAHDAYLNAVVGTALIKKYPKLESEFVYGDYKVYDVRKMIAKSEQEIGKATAKYFFYSNIMNFFKTEITLANGEIRKRPLIETNGETGEIVWDKGRDFATVRKVLSMPQVNIVKKTEVQTGGFSKESILPKRNSDKLIARKKDWDPKKYGGFDSPTVAYSVLVVAKVEKGKSKKLKSVKELLGITIMERSSFEKNPIDFLEAKGYKEVKKDLIIKLPKYSLFELENGRKRMLASAGELQKGNELALPSKYVNFLYLASHYEKLKGSPEDNEQKQLFVEQHKHYLDEIIEQISEFSKRVILADANLDKVLSAYNKHRDKPIREQAENIIHLFTLTNLGAPAAFKYFDTTIDRKRYTSTKEVLDATLIHQSITGLYETRIDLSQLGGDGSPKKKRKVSSDYKDHDGDYKDHDIDYKDDDDKAAGGGGSLPTCSCLDRVIQKDKGPYYTHLGAGPSVAAVREIMENRYGQKGNAIRIEIVVYTGKEGKSSHGCPIAKWVLRRSSDEEKVLCLVRQRTGHHCPTAVMVVLIMVWDGIPLPMADRLYTELTENLKSYNGHPTDRRCTLNENRTCTCQGIDPETCGASFSFGCSWSMYFNGCKFGRSPSPRRFRIDPSSPLHEKNLEDNLQSLATRLAPIYKQYAPVAYQNQVEYENVARECRLGSKEGRPFSGVTACLDFCAHPHRDIHNMNNGSTVVCTLTREDNRSLGVIPQDEQLHVLPLYKLSDTDEFGSKEGMEAKIKSGAIEVLAPRRKKRTCFTQPVPRSGKKRAAMMTEVLAHKIRAVEKKPIPRIKRKNNSTTTNNSKPSSLPTLGSNTETVQPEVKSETEPHFILKSSDNTKTYSLMPSAPHPVKEASPGFSWSPKTASATPAPLKNDATASCGFSERSSTPHCTMPSGRLSGANAAAADGPGISQLGEVAPLPTLSAPVMEPLINSEPSTGVTEPLTPHQPNHQPSFLTSPQDLASSPMEEDEQHSEADEPPSDEPLSDDPLSPAEEKLPHIDEYWSDSEHIFLDANIGGVAIAPAHGSVLIECARRELHATTPVEHPNRNHPTRLSLVFYQHKNLNKPQHGFELNKIKFEAKEAKNKKMKASEQKDQAANEGPEQSSEVNELNQIPSHKALTLTHDNVVTVSPYALTHVAGPYNHWV